European Patent Specification EP 3 137 100 B1, published December 20, 2023. Title: ISOLATED T CELL RECEPTORS AND METHODS OF USE THEREFOR. Applicant: University of Virginia Patent Foundation Zarling, Angela L Engelhard, Victor H Cummings, Kara Obeng, Rebecca. The sequence listing filed with the application follows.

SEQUENCE LISTING (55 sequences)

SEQ ID NO: 1 - protein, 1338 aa, Homo sapiens
MASPPRHGPPGPASGDGPNLNNNNNNNNHSVRKCGYLRKQKHGHKRFFVLRGPGAGGDEATAGGGSAPQPPRLEYYESEKKWRSKAGAPKRVIALDCCLNINKRADAKHKYLIALYTKDEYFAVAAENEQEQEGWYRALTDLVSEGRAAAGDAPPAAAPAASCSASLPGALGGSAGAAGAEDSYGLVAPATAAYREVWQVNLKPKGLGQSKNLTGVYRLCLSARTIGFVKLNCEQPSVTLQLMNIRRCGHSDSFFFIEVGRSAVTGPGELWMQADDSVVAQNIHETILEAMKALKELFEFRPRSKSQSSGSSATHPISVPGARRHHHLVNLPPSQTGLVRRSRTDSLAATPPAAKCSSCRVRTASEGDGGAAAGAAAAGARPVSVAGSPLSPGPVRAPLSRSHTLSGGCGGRGSKVALLPAGGALQHSRSMSMPVAHSPPAATSPGSLSSSSGHGSGSYPPPPGPHPPLPHPLHHGPGQRPSSGSASASGSPSDPGFMSLDEYGSSPGDLRAFCSHRSNTPESIAETPPARDGGGGGEFYGYMTMDRPLSHCGRSYRRVSGDAAQDLDRGLRKRTYSLTTPARQRPVPQPSSASLDEYTLMRATFSGSAGRLCPSCPASSPKVAYHPYPEDYGDIEIGSHRSSSSNLGADDGYMPMTPGAALAGSGSGSCRSDDYMPMSPASVSAPKQILQPRAAAAAAAAVPSAGPAGPAPTSAAGRTFPASGGGYKASSPAESSPEDSGYMRMWCGSKLSMEHADGKLLPNGDYLNVSPSDAVTTGTPPDFFSAALHPGGEPLRGVPGCCYSSLPRSYKAPYTCGGDSDQYVLMSSPVGRILEEERLEPQATPGPSQAASAFGAGPTQPPHPVVPSPVRPSGGRPEGFLGQRGRAVRPTRLSLEGLPSLPSMHEYPLPPEPKSPGEYINIDFGEPGARLSPPAPPLLASAASSSSLLSASSPASSLGSGTPGTSSDSRQRSPLSDYMNLDFSSPKSPKPGAPSGHPVGSLDGLLSPEASSPYPPLPPRPSASPSSSLQPPPPPPAPGELYRLPPASAVATAQGPGAASSLSSDTGDNGDYTEMAFGVAATPPQPIAAPPKPEAARVASPTSGVKRLSLMEQVSGVEAFLQASQPPDPHRGAKVIRADPQGGRRRHSSETFSSTTTVTPVSPSFAHNPKRHNSASVENVSLRKSSEGGVGVGPGGGDEPPTSPRQLQPAPPLAPQGRPWTPGQPGGLVGCPGSGGSPMRRETSAGFQNGLNYIAIDVREEPGLPPQPQPPPPPLPQPGDKSSWGRTRSLGGLISAVGVGSTGGGCGGPGPGALPPANTYASIDFLSHHLKEATIVKE

SEQ ID NO: 2 - protein, 9 aa, Homo sapiens
RVASPTSGV

SEQ ID NO: 3 - DNA, 807 bp, Mus musculus
  CDS (1)..(807)
atgctcctggcactcctcccagtgctggggatacactttgtcctgagagatgcccaagctcagtcagtgacacagcccgatgctcgcgtcactgtctctgaaggagcctctctgcagctgagatgcaagtattcctactctgggacgccttatctgttctggtatgtccagtacccgcggcaggggctgcagctgctcctcaagtactattccggagacccagtggttcaaggagtgaatggctttgaggctgagttcatcaagagtaactcttccttccacctgcggaaagcctctgtgcactggagcgactcggctgtgtacttctgtgctgtgagcgaaggtgcagatagactcacctttgggaaaggaactcagctgatcatccagccctacatccagaacccagaacctgctgtgtaccagttaaaagatcctcggtctcaggacagcaccctctgcctgttcaccgactttgactcccaaatcaatgtgccgaaaaccatggaatctggaacgctcatcactgacaaaactgtgctggacatgaaagctatggattccaagagcaatggggccattgcctggagcaaccagacaagcttcacctgccaagatatcttcaaagagaccaacgccacctaccccagttcagacgttccctgtgatgccacgttgactgagaaaagctttgaaacagatatgaacctaaactttcaaaacctgtcagttatgggactccgaatcctcctgctgaaagtagccggatttaacctgctcatgacgctgaggctgtggtccagttaa

SEQ ID NO: 4 - protein, 268 aa, Mus musculus
MLLALLPVLGIHFVLRDAQAQSVTQPDARVTVSEGASLQLRCKYSYSGTPYLFWYVQYPRQGLQLLLKYYSGDPVVQGVNGFEAEFIKSNSSFHLRKASVHWSDSAVYFCAVSEGADRLTFGKGTQLIIQPYIQNPEPAVYQLKDPRSQDSTLCLFTDFDSQINVPKTMESGTLITDKTVLDMKAMDSKSNGAIAWSNQTSFTCQDIFKETNATYPSSDVPCDATLTEKSFETDMNLNFQNLSVMGLRILLLKVAGFNLLMTLRLWSS

SEQ ID NO: 5 - DNA, 921 bp, Mus musculus
  CDS (1)..(921)
atgggcaccaggcttcttggctgggcagtgttctgtctccttgacacagtactgtctgaagctggagtcacccagtctcccagatatgcagtcctacaggaagggcaagctgtttccttttggtgtgaccctatttctggacatgataccctttactggtatcagcagcccagagaccaggggccccagcttctagtttactttcgggatgaggctgttatagataattcacagttgccctcggatcgattttctgctgtgaggcctaaaggaactaactccactctcaagatccagtctgcaaagcagggcgacacagccacctatctctgtgccagcagtttattggacagctcctatgaacagtacttcggtcccggcaccaggctcacggttttagaggatctgagaaatgtgactccacccaaggtctccttgtttgagccatcaaaagcagagattgcaaacaaacaaaaggctaccctcgtgtgcttggccaggggcttcttccctgaccacgtggagctgagctggtgggtgaatggcaaggaggtccacagtggggtcagcacggaccctcaggcctacaaggagagcaattatagctactgcctgagcagccgcctgagggtctctgctaccttctggcacaatcctcgaaaccacttccgctgccaagtgcagttccatgggctttcagaggaggacaagtggccagagggctcacccaaacctgtcacacagaacatcagtgcagaggcctggggccgagcagactgtggaatcacttcagcatcctatcatcagggggttctgtctgcaaccatcctctatgagatcctactggggaaggccaccctatatgctgtgctggtcagtggcctggtgctgatggccatggtcaagaaaaaaaattcctag

SEQ ID NO: 6 - protein, 306 aa, Mus musculus
MGTRLLGWAVFCLLDTVLSEAGVTQSPRYAVLQEGQAVSFWCDPISGHDTLYWYQQPRDQGPQLLVYFRDEAVIDNSQLPSDRFSAVRPKGTNSTLKIQSAKQGDTATYLCASSLLDSSYEQYFGPGTRLTVLEDLRNVTPPKVSLFEPSKAEIANKQKATLVCLARGFFPDHVELSWWVNGKEVHSGVSTDPQAYKESNYSYCLSSRLRVSATFWHNPRNHFRCQVQFHGLSEEDKWPEGSPKPVTQNISAEAWGRADCGITSASYHQGVLSATILYEILLGKATLYAVLVSGLVLMAMVKKKNS

SEQ ID NO: 7 - DNA, 810 bp, Mus musculus
  CDS (1)..(810)
atgctcctggcactcctcccagtgctggggatacactttgtcctgagagatgcccaagctcagtcagtgacacagcccgatgctcgcgtcactgtctctgaaggagcctctctgcagctgagatgcaagtattcctactctgggacgccttatctgttctggtatgtccagtacccgcggcaggggctgcagctgctcctcaagtactattccggagacccagtggttcaaggagtgaatggctttgaggctgagttcatcaagagtaactcttccttccacctgcggaaagcctctgtgcactggagcgactcggctgtgtacttctgtgctgtgagcgctggcagtggtggaaaactcactttgggggctggaacaagacttcaggtcaaccttgacatccagaacccagaacctgctgtgtaccagttaaaagatcctcggtctcaggacagcaccctctgcctgttcaccgactttgactcccaagtcaatgtgccgaaaaccatggaatctggaacgttcatcgctgacaaaactgtgctggacatgaaagctatggattccaagagcaatggggccattgcctggagcaaccagacaagcttcacctgccaagatatcttcaaagagaccaacgccacctaccccagttcagacgttccctgtgatgccacgttgactgagaaaagctttgaaacagatatgaacctaaactttcaaaacctgtcagttatgggactccgaatcctcctgctgaaagtagccggatttaacctgctcatgacgctgaggctgtggtccagttaa

SEQ ID NO: 8 - protein, 269 aa, Mus musculus
MLLALLPVLGIHFVLRDAQAQSVTQPDARVTVSEGASLQLRCKYSYSGTPYLFWYVQYPRQGLQLLLKYYSGDPVVQGVNGFEAEFIKSNSSFHLRKASVHWSDSAVYFCAVSAGSGGKLTLGAGTRLQVNLDIQNPEPAVYQLKDPRSQDSTLCLFTDFDSQVNVPKTMESGTFIADKTVLDMKAMDSKSNGAIAWSNQTSFTCQDIFKETNATYPSSDVPCDATLTEKSFETDMNLNFQNLSVMGLRILLLKVAGFNLLMTLRLWSS

SEQ ID NO: 9 - DNA, 915 bp, Mus musculus
  CDS (1)..(915)
atgggctccagactcttctttgtggttttgattctcctgtgtgcaaaacacatggaggctgcagtcacccaaagtccaagaagcaaggtggcagtaacaggaggaaaggtgacattgagctgtcaccaggctaataaccatgactatatgtactggtatcggcaggacacggggcatgggctgaggctgatccattactcatatgtcgctgacagcacggagaaaggagatatccctgatgggtacaaggcctccagaccaagccaagagaatttctctctcattctggagttggcttccctttctcagacagctgtatatttctgtgccagcagtgatagggacaactatgctgagcagttcttcggaccagggacacgactcaccgtcctagaggatctgagaaatgtgactccacccaaggtctccttgtttgagccatcaaaagcagagattgcaaacaaacaaaaggctaccctcgtgtgcttggccaggggcttcttccctgaccacgtggagctgagctggtgggtgaatggcaaggaggtccgcagtggggtcagcacggaccctcaggcctacaaggagagcaattatagctactgcctgagcagccgcctgagggtctctgctaccttctggcacaatcctcgaaaccacttccgctgccaagtgcagttccatgggctttcagaggaggacaagtggccagagggctcacccaaacctgtcacacagaacatcagtgcagaggcctggggccgagcagactgtggaatcacttcagcatcctatcatcagggggttctgtctgcaaccatcctctatgagatcctactggggaaggccaccctatacgctgtgctggtcagtggcctggtgctgatggccatggtcaagaaaaaaaattcctaa

SEQ ID NO: 10 - protein, 304 aa, Mus musculus
MGSRLFFVVLILLCAKHMEAAVTQSPRSKVAVTGGKVTLSCHQANNHDYMYWYRQDTGHGLRLIHYSYVADSTEKGDIPDGYKASRPSQENFSLILELASLSQTAVYFCASSDRDNYAEQFFGPGTRLTVLEDLRNVTPPKVSLFEPSKAEIANKQKATLVCLARGFFPDHVELSWWVNGKEVRSGVSTDPQAYKESNYSYCLSSRLRVSATFWHNPRNHFRCQVQFHGLSEEDKWPEGSPKPVTQNISAEAWGRADCGITSASYHQGVLSATILYEILLGKATLYAVLVSGLVLMAMVKKKNS

SEQ ID NO: 11 - protein, 580 aa, Homo sapiens
MEVPQPEPAPGSALSPAGVCGGAQRPGHLPGLLLGSHGLLGSPVRAAASSPVTTLTQTMHDLAGLGSETPKSQVGTLLFRSRSRLTHLSLSRRASESSLSSESSESSDAGLCMDSPSPMDPHMAEQTFEQAIQAASRIIRNEQFAIRRFQSMPVRLLGHSPVLRNITNSQAPDGRRKSEAGSGAASSSGEDKENDGFVFKMPWKPTHPSSTHALAEWASRREAFAQRPSSAPDLMCLSPDRKMEVEELSPLALGRFSLTPAEGDTEEDDGFVDILESDLKDDDAVPPGMESLISAPLVKTLEKEEEKDLVMYSKCQRLFRSPSMPCSVIRPILKRLERPQDRDTPVQNKRRRSVTPPEEQQEAEEPKARVLRSKSLCHDEIENLLDSDHRELIGDYSKAFLLQTVDGKHQDLKYISPETMVALLTGKFSNIVDKFVIVDCRYPYEYEGGHIKTAVNLPLERDAESFLLKSPIAPCSLDKRVILIFHCEFSSERGPRMCRFIRERDRAVNDYPSLYYPEMYILKGGYKEFFPQHPNFCEPQDYRPMNHEAFKDELKTFRLKTRSWAGERSRRELCSRLQDQ

SEQ ID NO: 12 - protein, 9 aa, Homo sapiens
GLLGSPVRA

SEQ ID NO: 13 - DNA, 810 bp, Mus musculus
  CDS (1)..(810)
atgaagacagtgactggacctttgttcctgtgcttctggctgcagctgaactgtgtgagcagaggcgagcaggtggagcagcgccctcctcacctgagtgtccgggagggagacagtgccgttatcatctgcacctacacagaccctaacagttattacttcttctggtacaagcaagagccgggggcaggtcttcagttgcttatgaaggttttctcaagtacggaaataaacgaagggcaaggattcactgtcctactgaacaagaaagaccaacaactctctctgaacctcacagctgcccatcctggggactcagccgtgtacttctgcgcagtcaaacctggaggctataaagtggtctttggaagtgggactcgattgctggtaagccctgacatccagaacccagaacctgctgtgtaccagttaaaagatcctcggtctcaggacagcaccctctgcctgttcaccgactttgactcccaaatcaatgtgccgaaaaccatggaatctggaacgttcatcactgacaaaactgtgctggacatgaaagctatggattccaagagcaatggggccattgcctggagcaaccagacaagcttcacctgccaagatatcttcaaagagaccaacgccacctaccccagttcagacgttccctgtgatgccacgttgacagagaaaagctttgaaacagatatgaacctaaactttcaaaacctgtcagttatgggactccgaatcctcctgctgaaagtagccggatttaacctgctcatgacgctgaggctgtggtccagttaa

SEQ ID NO: 14 - protein, 269 aa, Mus musculus
MKTVTGPLFLCFWLQLNCVSRGEQVEQRPPHLSVREGDSAVIICTYTDPNSYYFFWYKQEPGAGLQLLMKVFSSTEINEGQGFTVLLNKKDQQLSLNLTAAHPGDSAVYFCAVKPGGYKVVFGSGTRLLVSPDIQNPEPAVYQLKDPRSQDSTLCLFTDFDSQINVPKTMESGTFITDKTVLDMKAMDSKSNGAIAWSNQTSFTCQDIFKETNATYPSSDVPCDATLTEKSFETDMNLNFQNLSVMGLRILLLKVAGFNLLMTLRLWSS

SEQ ID NO: 15 - DNA, 936 bp, Mus musculus
  CDS (1)..(936)
atgtctaacactgccttccctgaccccgcctggaacaccaccctgctatcttgggttgctctctttctcctgggaacaaaacacatggaggctgcagtcacccaaagcccaagaaacaaggtggcagtaacaggaggaaaggtgacattgagctgtaatcagactaataaccacaacaacatgtactggtatcggcaggacacggggcatgggctgaggctgatccattattcatatggtgctggcagcactgagaaaggagatatccctgatggatacaaggcctccagaccaagccaagagaacttctccctcattctggagttggctaccccctctcagacatcagtgtacttctgtgccagcggtggcgacacccagtactttgggccaggcactcggctcctcgtgttagaggatctgagaaatgtgactccacccaaggtctccttgtttgagccatcaaaagcagagattgcaaacaaacaaaaggctaccctcgtgtgcttggccaggggcttcttccctgaccacgtggagctgagctggtgggtgaatggcaaggaggtccacagtggggtcagcacggaccctcaggcctacaaggagcgcaattatagctactgcctgagcagccgcctgagggtctctgctaccttctggcacaatcctcgaaaccacttccgctgccaagtgcagttccatgggctttcagaggaggacaagtggccagagggctcacccaaacctgtcacacagaacatcagtgcagaggcctggggccgagcagactgtggaatcacttcagcatcctatcatcagggggttctgtctgcaaccatcctctatgagatcctactggggaaggccaccctatatgctgtgctggtcagtggcctggtgctgatggccatggtcaagaaaaaaaattcctaa

SEQ ID NO: 16 - protein, 311 aa, Mus musculus
MSNTAFPDPAWNTTLLSWVALFLLGTKHMEAAVTQSPRNKVAVTGGKVTLSCNQTNNHNNMYWYRQDTGHGLRLIHYSYGAGSTEKGDIPDGYKASRPSQENFSLILELATPSQTSVYFCASGGDTQYFGPGTRLLVLEDLRNVTPPKVSLFEPSKAEIANKQKATLVCLARGFFPDHVELSWWVNGKEVHSGVSTDPQAYKERNYSYCLSSRLRVSATFWHNPRNHFRCQVQFHGLSEEDKWPEGSPKPVTQNISAEAWGRADCGITSASYHQGVLSATILYEILLGKATLYAVLVSGLVLMAMVKKKNS

SEQ ID NO: 17 - protein, 1565 aa, Homo sapiens
MLSWRLQTGPEKAELQELNARLYDYVCRVRELERENLLLEEELRGRRGREGLWAEGQARCAEEARSLRQQLDELSWATALAEGERDALRRELRELQRLDAEERAARGRLDAELGAQQRELQEALGARAALEALLGRLQAERRGLDAAHERDVRELRARAASLTMHFRARATGPAAPPPRLREVHDSYALLVAESWRETVQLYEDEVRELEEALRRGQESRLQAEEETRLCAQEAEALRREALGLEQLRARLEDALLRMREEYGIQAEERQRVIDCLEDEKATLTLAMADWLRDYQDLLQVKTGLSLEVATYRALLEGESNPEIVIWAEHVENMPSEFRNKSYHYTDSLLQRENERNLFSRQKAPLASFNHSSALYSNLSGHRGSQTGTSIGGDARRGFLGSGYSSSATTQQENSYGKAVSSQTNVRTFSPTYGLLRNTEAQVKTFPDRPKAGDTREVPVYIGEDSTIARESYRDRRDKVAAGASESTRSNERTVILGKKTEVKATREQERNRPETIRTKPEEKMFDSKEKASEERNLRWEELTKLDKEARQRESQQMKEKAKEKDSPKEKSVREREVPISLEVSQDRRAEVSPKGLQTPVKDAGGGTGREAEARELRFRLGTSDATGSLQGDSMTETVAENIVTSILKQFTQSPETEASADSFPDTKVTYVDRKELPGERKTKTEIVVESKLTEDVDVSDEAGLDYLLSKDIKEVGLKGKSAEQMIGDIINLGLKGREGRAKVVNVEIVEEPVSYVSGEKPEEFSVPFKVEEVEDVSPGPWGLVKEEEGYGESDVTFSVNQHRRTKQPQENTTHVEEVTEAGDSEGEQSYFVSTPDEHPGGHDRDDGSVYGQIHIEEESTIRYSWQDEIVQGTRRRTQKDGAVGEKVVKPLDVPAPSLEGDLGSTHWKEQARSGEFHAEPTVIEKEIKIPHEFHTSMKGISSKEPRQQLVEVIGQLEETLPERMREELSALTREGQGGPGSVSVDVKKVQGAGGSSVTLVAEVNVSQTVDADRLDLEELSKDEASEMEKAVESVVRESLSRQRSPAPGSPDEEGGAEAPAAGIRFRRWATRELYIPSGESEVAGGASHSSGQRTPQGPVSATVEVSSPTGFAQSQVLEDVSQAARHIKLGPSEVWRTERMSYEGPTAEVVEVSAGGDLSQAASPTGASRSVRHVTLGPGQSPLSREVIFLGPAPACPEAWGSPEPGPAESSADMDGSGRHSTFGCRQFHAEKEIIFQGPISAAGKVGDYFATEESVGTQTSVRQLQLGPKEGFSGQIQFTAPLSDKVELGVIGDSVHMEGLPGSSTSIRHISIGPQRHQTTQQIVYHGLVPQLGESGDSESTVHGEGSADVHQATHSHTSGRQTVMTEKSTFQSVVSESPQEDSAEDTSGAEMTSGVSRSFRHIRLGPTETETSEHIAIRGPVSRTFVLAGSADSPELGKLADSSRTLRHIAPGPKETSFTFQMDVSNVEAIRSRTQEAGALGVSDRGSWRDADSRNDQAVGVSFKASAGEGDQAHREQGKEQAMFDKKVQLQRMVDQRSVISDEKKVALLYLDNEEEENDGHWF

SEQ ID NO: 18 - protein, 1253 aa, Homo sapiens
MLSWRLQTGPEKAELQELNARLYDYVCRVRELERENLLLEEELRGRRGREGLWAEGQARCAEEARSLRQQLDELSWATALAEGERDALRRELRELQRLDAEERAARGRLDAELGAQQRELQEALGARAALEALLGRLQAERRGLDAAHERDVRELRARAASLTMHFRARATGPAAPPPRLREVHDSYALLVAESWRETVQLYEDEVRELEEALRRGQESRLQAEEETRLCAQEAEALRREALGLEQLRARLEDALLRMREEYGIQAEERQRVIDCLEDEKATLTLAMADWLRDYQDLLQVKTGLSLEVATYRALLEGESNPEIVIWAEHVENMPSEFRNKSYHYTDSLLQRENERNLFSRQKAPLASFNHSSALYSNLSGHRGSQTGTSIGGDARRGFLGSGYSSSATTQQENSYGKAVSSQTNVRTFSPTYGLLRNTEAQVKTFPDRPKAGDTREVPVYIGEDSTIARESYRDRRDKVAAGASESTRSNERTVILGKKTEVKATREQERNRPETIRTKPEEKMFDSKEKASEERNLRWEELTKLDKEARQRESQQMKEKAKEKDSPKEKSVREREVPISLEVSQDRRAEVSPKGLQTPVKDAGGGTGREAEARELRFRLGTSDATGSLQGDSMTETVAENIVTSILKQFTQSPETEASADSFPDTKVTYVDRKELPGERKTKTEIVVESKLTEDVDVSDEAGLDYLLSKDIKEVGLKGKSAEQMIGDIINLGLKGREGRAKVVNVEIVEEPVSYVSGEKPEEFSVPFKVEEVEDVSPGPWGLVKEEEGYGESDVTFSVNQHRRTKQPQENTTHVEEVTEAGDSEGEQSYFVSTPDEHPGGHDRDDGSVYGQIHIEEESTIRYSWQDEIVQGTRRRTQKDGAVGEKVVKPLDVPAPSLEGDLGSTHWKEQARSGEFHAEPTVIEKEIKIPHEFHTSMKGISSKEPRQQLVEVIGQLEETLPERMREELSALTREGQGGPGSVSVDVKKVQGAGGSSVTLVAEVNVSQTVDADRLDLEELSKDEASEMEKAVESVVRESLSRQRSPAPGSPDEEGGAEAPAAGIRFRRWATRELYIPSGESEVAGGASHSSGQRTPQGPVSATVEVSSPTGFAQSQVLEDVSQAARHIKLGPSEVWRTERMSYEGPTAEVVEMDVSNVEAIRSRTQEAGALGVSDRGSWRDADSRNDQAVGVSFKASAGEGDQAHREQGKEQAMFDKKVQLQRMVDQRSVISDEKKVALLYLDNEEEENDGHWF

SEQ ID NO: 19 - protein, 9 aa, Homo sapiens
RTFSPTYGL

SEQ ID NO: 20 - DNA, 807 bp, Mus musculus
  CDS (1)..(807)
atgctcctggcgctcctcccagtgctggggatacactttgtcctgagagatgcccaagctcagtcagtgacgcagcccgatgctcgcgccactgtctctgaaggagcctctctgcggctgagatgcaagtattcctactctgggacaccttatctgttctggtatgtccagtacccgcggcaggggctgcagctgctcctcaagtactattcaggagacccagtggttcaaggagtgaatggcttcgaggctgagttcagcaagagtaactcttccttccacctgcggaaagcctctgtgcactggagcgactctgctgtgtacttctgtgttttgagctatagcaataacagaatcttctttggtgatgggacgcagctggtgatgaagcccaacatccagaacccagaacctgctgtgtaccagttaaaagatcctcggtctcaggacagcaccctctgcctgttcaccgactttgactcccaaatcaatgtgccgaaaaccatggaatctggaacgttcatcactgacaaaactgtgctggacatgaaagctatggattccaagagcaatggggccattgcctggagcaaccagacaagcttcacctgccaagatatcttcaaagagaccaacgccacctaccccagttcagacgttccctgtgatgccacgttgactgagaaaagctttgaaacagatatgaacctaaactttcaaaacctgtcagttatgggactccgaatcctcctgctgaaagtagccggatttaacctgctcatgacgctgaggctgtggtccagttaa

SEQ ID NO: 21 - protein, 268 aa, Mus musculus
MLLALLPVLGIHFVLRDAQAQSVTQPDARATVSEGASLRLRCKYSYSGTPYLFWYVQYPRQGLQLLLKYYSGDPVVQGVNGFEAEFSKSNSSFHLRKASVHWSDSAVYFCVLSYSNNRIFFGDGTQLVMKPNIQNPEPAVYQLKDPRSQDSTLCLFTDFDSQINVPKTMESGTFITDKTVLDMKAMDSKSNGAIAWSNQTSFTCQDIFKETNATYPSSDVPCDATLTEKSFETDMNLNFQNLSVMGLRILLLKVAGFNLLMTLRLWSS

SEQ ID NO: 22 - DNA, 942 bp, Mus musculus
  CDS (1)..(942)
  misc_feature (582)..(583): n is a, c, g, or t
atgtctaacactgtcctcgctgattctgcctggggcatcaccctgctatcttgggttactgtctttctcttgggaacaagttcagcagattctggggttgtccagtctccaagacacataatcaaagaaaagggaggaaggtccgttctgacgtgtattcccatctctggacatagcaatgtggtctggtaccagcagactctggggaaggaattaaagttccttattcagcattatgaaaaggtggagagagacaaaggattcctacccagcagattctcagtccaacagtttgatgactatcactctgaaatgaacatgagtgccttggaactggaggactctgctatgtacttctgtgccagctctctggggggtggagaagtcttctttggtaaaggaaccagactcacagttgtagaggatctgagaaatgtgactccacccaaggtctccttgtttgagccatcaaaagcagagattgcaaacaaacaaaaggctaccctcgtgtgcttggccaggggcttcttccctgaccacgtggagctgagctggtgggtgaatggcaaggaggtccacagnngggtcagcacggaccctcaggcctacaaggagagcaattatagctactgcctgagcagccgcctgagggtctctgctaccttctggcacaatcctcgcaaccacttccgctgccaagtgcagttccatgggctttcagaggaggacaagtggccagagggctcacccaaacctgtcacacagaacatcagtgcagaggcctggggccgagcagactgtgggattacctcagcatcctatcaacaaggggtcttgtctgccaccatcctctatgagatcctgctagggaaagccaccctgtatgctgtgcttgtcagtacactggtggtgatggctatggtcaaaaaaaagaattcctaa

SEQ ID NO: 23 - protein, 313 aa, Mus musculus
  misc_feature (194)..(194): The 'Xaa' at location 194 stands for Arg, or Ser.
  misc_feature (195)..(195): The 'Xaa' at location 195 stands for Arg, Gly, or Trp.
MSNTVLADSAWGITLLSWVTVFLLGTSSADSGVVQSPRHIIKEKGGRSVLTCIPISGHSNVVWYQQTLGKELKFLIQHYEKVERDKGFLPSRFSVQQFDDYHSEMNMSALELEDSAMYFCASSLGGGEVFFGKGTRLTVVEDLRNVTPPKVSLFEPSKAEIANKQKATLVCLARGFFPDHVELSWWVNGKEVHXXVSTDPQAYKESNYSYCLSSRLRVSATFWHNPRNHFRCQVQFHGLSEEDKWPEGSPKPVTQNISAEAWGRADCGITSASYQQGVLSATILYEILLGKATLYAVLVSTLVVMAMVKKKNS

SEQ ID NO: 24 - DNA, 810 bp, Mus musculus
  CDS (1)..(810)
atgctcctggcgctcctcccagtgctggggatacactttgtcctgagagatgcccaagctcagtcagtgacgcagcccgatgctcgcgtcactgtctctgaaggagcctctctgcagctgagatgcaagtattcctactctgggacaccttatctgttctggtatgcccagtacccgcggcaggggctgcagctgctcctcaagtactattcaggagacccagtggttcaaggagtgaatggcttcgaggctgagttcagcaagagtaactcttccttccacctgcggaaagcctctgtgcactggagcgactctgctgtgtacttctgtgttttgaggtacggaggcaataataagctgacttttggtcaaggaaccgttctgagtgttataccagacatccagaacccagaacctgctgtgtaccagttaaaagatcctcggtctcaggacagcaccctctgcctgttcaccgactttgactcccaaatcaatgtgccgaaaaccatggaatctggaacgttcatcactgacaaaactgtgctggacatgaaagctatggattccaagagcaatggggccattgcctggagcaaccagacaagcttcacctgccaagatatcttcaaagagaccaacgccacctaccccagttcagacgttccctgtgatgccacgttgactgagaaaagctttgaaacagatatgaacctaaactttcagaacctgtcagttatgggactccgaatcctcctgctgaaagtagccggatttaacctgctcatgacgctgaggctgtggtccagttga

SEQ ID NO: 25 - protein, 269 aa, Mus musculus
MLLALLPVLGIHFVLRDAQAQSVTQPDARVTVSEGASLQLRCKYSYSGTPYLFWYAQYPRQGLQLLLKYYSGDPVVQGVNGFEAEFSKSNSSFHLRKASVHWSDSAVYFCVLRYGGNNKLTFGQGTVLSVIPDIQNPEPAVYQLKDPRSQDSTLCLFTDFDSQINVPKTMESGTFITDKTVLDMKAMDSKSNGAIAWSNQTSFTCQDIFKETNATYPSSDVPCDATLTEKSFETDMNLNFQNLSVMGLRILLLKVAGFNLLMTLRLWSS

SEQ ID NO: 26 - DNA, 906 bp, Mus musculus
  CDS (1)..(906)
atgggctccagactcttctttgtggttttgattctcctgtgtgcaaaacacatggaggctgcagtcacccaaagtccaagaagcaaggtggcggtaacaggaggaaaggtgacattgagctgtcaccagactaataaccatgactatatgtactggtatcggcaggacacggggcatgggctgaggctgatccattactcatatgtcgctgacagcacggagaaaggagatatccctgatgggtacaaggcctccagaccaagccaagagaatttctctctcattctggagttggcttccctttctcagacagctgtatatttctgtgccagcaggtacagggacacccagtactttgggccaggcactcggctcctcgtgttagaggatctgagaaatgtgactccacccaaggtctccttgtttgagccatcaaaagcagagattgcaaacaagcaaaaggctaccctcgtgtgcttggccaggggcttcttccctgaccacgtggagctgagctggtgggtgaatggcaaggaggtccacagtggggtcagcacggaccctcaggcctacaaggagagcaattatagctactgcctgagcagccgcctgagggtctctgctaccttctggcacaatcctcgaaaccacttccgctgccaagtgcagttccatgggctttcagaggaggacaagtggccagagggctcacccaaacctgtcacacagaacatcagtgcagaggcctggggccgagcagactgtggaatcacttcagcatcctatcatcagggggttctgtctgcaaccatcctctatgagatcctactggggaaggccaccctatatgctgtgctggtcagtggcctggtgctgatggccatggtcaagaaaaaaaattcctag

SEQ ID NO: 27 - protein, 301 aa, Mus musculus
MGSRLFFVVLILLCAKHMEAAVTQSPRSKVAVTGGKVTLSCHQTNNHDYMYWYRQDTGHGLRLIHYSYVADSTEKGDIPDGYKASRPSQENFSLILELASLSQTAVYFCASRYRDTQYFGPGTRLLVLEDLRNVTPPKVSLFEPSKAEIANKQKATLVCLARGFFPDHVELSWWVNGKEVHSGVSTDPQAYKESNYSYCLSSRLRVSATFWHNPRNHFRCQVQFHGLSEEDKWPEGSPKPVTQNISAEAWGRADCGITSASYHQGVLSATILYEILLGKATLYAVLVSGLVLMAMVKKKNS

SEQ ID NO: 28 - protein, 781 aa, Homo sapiens
MATQADLMELDMAMEPDRKAAVSHWQQQSYLDSGIHSGATTTAPSLSGKGNPEEEDVDTSQVLYEWEQGFSQSFTQEQVADIDGQYAMTRAQRVRAAMFPETLDEGMQIPSTQFDAAHPTNVQRLAEPSQMLKHAVVNLINYQDDAELATRAIPELTKLLNDEDQVVVNKAAVMVHQLSKKEASRHAIMRSPQMVSAIVRTMQNTNDVETARCTAGTLHNLSHHREGLLAIFKSGGIPALVKMLGSPVDSVLFYAITTLHNLLLHQEGAKMAVRLAGGLQKMVALLNKTNVKFLAITTDCLQILAYGNQESKLIILASGGPQALVNIMRTYTYEKLLWTTSRVLKVLSVCSSNKPAIVEAGGMQALGLHLTDPSQRLVQNCLWTLRNLSDAATKQEGMEGLLGTLVQLLGSDDINVVTCAAGILSNLTCNNYKNKMMVCQVGGIEALVRTVLRAGDREDITEPAICALRHLTSRHQEAEMAQNAVRLHYGLPVVVKLLHPPSHWPLIKATVGLIRNLALCPANHAPLREQGAIPRLVQLLVRAHQDTQRRTSMGGTQQQFVEGVRMEEIVEGCTGALHILARDVHNRIVIRGLNTIPLFVQLLYSPIENIQRVAAGVLCELAQDKEAAEAIEAEGATAPLTELLHSRNEGVATYAAAVLFRMSEDKPQDYKKRLSVELTSSLFRTEPMAWNETADLGLDIGAQGEPLGYRQDDPSYRSFHSGGYGQDALGMDPMMEHEMGGHHPGADYPVDGLPDLGHAQDLMDGLPPGDSNQLAWFDTDL

SEQ ID NO: 29 - protein, 10 aa, Homo sapiens
YLDSGIHSGV

SEQ ID NO: 30 - protein, 10 aa, Homo sapiens
YLDSGIHSGA

SEQ ID NO: 31 - DNA, 801 bp, Mus musculus
  CDS (1)..(801)
atgaagaggctgctgtgttctctgctggggcttctgtgcacccaggtttgctgggtgaaaggacagcaagtgcagcagagtcccgcatccttggttctgcaggagggggagaacgcagagctgcagtgtaacttttcctccacagcaacccggctgcagtggttttaccaacatcctgggggaagactcgtcagcctgttctacaatccttctgggacaaagcacactggaagactgacatccaccacagtcactaacgaacgtcgcagctctttgcacatttcctcctcccagacaacagactcaggcacttatttctgtgctatccccccaggcactgggtctaagctgtcatttgggaagggggcaaagctcacagtgagtccagacatccagaacccagaacctgctgtgtaccagttaaaagatcctcggtctcaggacagcaccctctgcctgttcaccgactttgactcccaaatcaatgtgccgaaaaccatggaatctggaacgttcatcactgacaaaactgtgctggacatgaaagctatggattccaagagcaatggggccattgcctggagcaaccagacaagcttcacctgccaagatatcttcaaagagaccaacgccacctaccccagttcagacgttccctgtgatgccacgttgactgagaaaagctttgaaacagatatgaacctaaactttcaaaacctgtcagttatgggactccgaatcctcctgctgaaagtagccggatttaacctgctcatgacgctgaggctgtggtccagttaa

SEQ ID NO: 32 - protein, 266 aa, Mus musculus
MKRLLCSLLGLLCTQVCWVKGQQVQQSPASLVLQEGENAELQCNFSSTATRLQWFYQHPGGRLVSLFYNPSGTKHTGRLTSTTVTNERRSSLHISSSQTTDSGTYFCAIPPGTGSKLSFGKGAKLTVSPDIQNPEPAVYQLKDPRSQDSTLCLFTDFDSQINVPKTMESGTFITDKTVLDMKAMDSKSNGAIAWSNQTSFTCQDIFKETNATYPSSDVPCDATLTEKSFETDMNLNFQNLSVMGLRILLLKVAGFNLLMTLRLWSS

SEQ ID NO: 33 - DNA, 906 bp, Mus musculus
  CDS (1)..(906)
atgagctgcaggcttctcctctatgtttccctatgtcttgtggaaacagcactcatgaacactaaaattactcagtcaccaagatatctaatcctgggaagagcaaataagtctttggaatgtgagcaacatctgggacataatgctatgtactggtataaacagagcgctgagaagccgccagagctcatgtttctctacaatcttaaacagttgattcgaaatgagacggtgcccagtcgttttatacctgaatgcccagacagctccaagctacttttacatatatctgccgtggatccagaagactcagctgtctatttttgtgccagcagccaaggacagaaacagtacttcggtcccggcaccaggctcacggttttagaggatctgagaaatgtgactccacccaaggtctccttgtttgagccatcaaaagcagagattgcaaacaaacaaaaggctaccctcgtgtgcttggccaggggcttcttccctgaccacgtggagctgagctggtgggtgaatggcaaggaggtccacagtggggtcagcacggaccctcaggcctacaaggagagcaattatagctactgcctgagcagccgcctgagggtctctgctaccttctggcacaatcctcgaaaccacttccgctgccaagtgcagttccatgggctttcagaggaggacaagtggccagagggcttacccaaacctgtcacacagaacatcagtgcagaggcctggggccgagcagactgtggaatcacttcagcatcctatcatcagggggttctgtctgcaaccatcctctatgagatcctactggggaaggccaccctatatgctgtgctggtcagtggcctggtgctgatggccatggtcaagaaaaaaaattcctaa

SEQ ID NO: 34 - protein, 301 aa, Mus musculus
MSCRLLLYVSLCLVETALMNTKITQSPRYLILGRANKSLECEQHLGHNAMYWYKQSAEKPPELMFLYNLKQLIRNETVPSRFIPECPDSSKLLLHISAVDPEDSAVYFCASSQGQKQYFGPGTRLTVLEDLRNVTPPKVSLFEPSKAEIANKQKATLVCLARGFFPDHVELSWWVNGKEVHSGVSTDPQAYKESNYSYCLSSRLRVSATFWHNPRNHFRCQVQFHGLSEEDKWPEGLPKPVTQNISAEAWGRADCGITSASYHQGVLSATILYEILLGKATLYAVLVSGLVLMAMVKKKNS

SEQ ID NO: 35 - DNA, 804 bp, Mus musculus
  CDS (1)..(804)
atgaacagattcctgggaatatctttggtgactctatggtttcaagtggcctgggcaaagagccaatggggagaagagaatcttcaggctctgagcatccaggagggtgaagatgtcaccatgaactgcagttacaagacttacacaactgttgttcagtggtacagacagaagtcaggcaaaggccctgcccagctaatcttaatacgttcaaatgagcgagagaagcgcagtggaagactcagagccacccttgacacttccagccagagcagctccctgtccatcactggtactctagctacagacactgctgtgtacttctgtgctactgggcccaataccaacaaagtcgtctttggaacagggaccagattacaagtattaccaaacatccagaacccagaacctgctgtgtaccagttaaaagatcctcggtctcaggacagcaccctctgcctgttcaccgactttgactcccaaatcaatgtgccgaaaaccatggaatctggaacgttcatcactgacaaaactgtgctggacatgaaagctatggattccaagagcaatggggccattgcctggagcaaccagacaagcttcacctgccaagatatcttcaaagagaccaacgccacctaccccagttcagacgttccctgtgatgccacgttgactgagaaaagctttgaaacagatatgaacctaaactttcaaaacctgtcagttatgggactccgaatcctcctgctgaaagtagccggatttaacctgctcatgacgctgaggctgtggtccagttga

SEQ ID NO: 36 - protein, 267 aa, Mus musculus
MNRFLGISLVTLWFQVAWAKSQWGEENLQALSIQEGEDVTMNCSYKTYTTVVQWYRQKSGKGPAQLILIRSNEREKRSGRLRATLDTSSQSSSLSITGTLATDTAVYFCATGPNTNKVVFGTGTRLQVLPNIQNPEPAVYQLKDPRSQDSTLCLFTDFDSQINVPKTMESGTFITDKTVLDMKAMDSKSNGAIAWSNQTSFTCQDIFKETNATYPSSDVPCDATLTEKSFETDMNLNFQNLSVMGLRILLLKVAGFNLLMTLRLWSS

SEQ ID NO: 37 - DNA, 909 bp, Mus musculus
  CDS (1)..(909)
atgagctgcaggcttctcctctatgtttccctatgtcttgtggaaacagcactcatgaacactaaaattactcagtcaccaagatatctaatcctgggaagagcaaataagtctttggaatgtgagcaacatctgggacataatgctatgtactggtataaacagagcgctgagaagccgccagagctcatgtttctctacaatcttaaacagttgattcgaaatgagacggtgcccagtcgttttatacctgaatgcccagacagctccaagctacttttacatatatctgccgtggatccagaagactcagctgtctatttttgtgccagcagccaaggtggtgctgagcagttcttcggaccagggacacgactcaccgtcctagaggatctgagaaatgtgactccacccaaggtctccttgtttgagccatcaaaagcagagattgcaaacaaacaaaaggctaccctcgtgtgcttggccaggggcttcttccctgaccacgtggagctgagctggtgggtgaatggcaaggaggtccacagtggggtcagcacggaccctcaggcctacaaggagagcaattatagctactgcctgagcagccgcctgagggtctctgctaccttctggcacaatcctcgaaaccacttccgctgccaagtgcagttccatgggctttcagaggaggacaagtggccagagggctcacccaaacctgtcacacagaacatcagtgcagaggcctggggccgagcagactgtggaatcacttcagcatcctatcatcagggggttctgtctgcaaccatcctctatgagatcctactggggaaggccaccctatatgctgtgctggtcagtggcctggtgctgatggccatggtcaagaaaaaaaattcctag

SEQ ID NO: 38 - protein, 302 aa, Mus musculus
MSCRLLLYVSLCLVETALMNTKITQSPRYLILGRANKSLECEQHLGHNAMYWYKQSAEKPPELMFLYNLKQLIRNETVPSRFIPECPDSSKLLLHISAVDPEDSAVYFCASSQGGAEQFFGPGTRLTVLEDLRNVTPPKVSLFEPSKAEIANKQKATLVCLARGFFPDHVELSWWVNGKEVHSGVSTDPQAYKESNYSYCLSSRLRVSATFWHNPRNHFRCQVQFHGLSEEDKWPEGSPKPVTQNISAEAWGRADCGITSASYHQGVLSATILYEILLGKATLYAVLVSGLVLMAMVKKKNS

SEQ ID NO: 39 - DNA, 24 bp, Artificial sequence
  Artificially synthesized oligonucleotide primer
actggaccacagcctcagcgtcat

SEQ ID NO: 40 - DNA, 27 bp, Artificial sequence
  Artificially synthesized oligonucleotide primer
tgaattctttcttttgaccatagccat

SEQ ID NO: 41 - DNA, 27 bp, Artificial sequence
  Artificially synthesized oligonucleotide primer
ggaattttttttcttgaccatggccat

SEQ ID NO: 42 - DNA, 49 bp, Artificial sequence
  Artificially synthesized oligonucleotide primer
taatacgactcactatagggagagccaccatgctcctggcactcctccc

SEQ ID NO: 43 - DNA, 89 bp, Artificial sequence
  Artificially synthesized oligonucleotide primer
ttttttttttttttttttttttttttttttttttttttttttttttttttttttttttttttttttaactggaccacagcctcagcgtc

SEQ ID NO: 44 - DNA, 49 bp, Artificial sequence
  Artificially synthesized oligonucleotide primer
taatacgactcactatagggagagccaccatgggcaccaggcttcttgg

SEQ ID NO: 45 - DNA, 92 bp, Artificial sequence
  Artificially synthesized oligonucleotide primer
ttttttttttttttttttttttttttttttttttttttttttttttttttttttttttttttttttaggaattttttttcttgaccatggcc

SEQ ID NO: 46 - DNA, 49 bp, Artificial sequence
  Artificially synthesized oligonucleotide primer
taatacgactcactatagggagagccaccatgaagacagtgactggacc

SEQ ID NO: 47 - DNA, 50 bp, Artificial sequence
  Artificially synthesized oligonucleotide primer
taatacgactcactatagggagagccaccatgtctaacactgccttccct

SEQ ID NO: 48 - DNA, 50 bp, Artificial Sequence
  Artificially synthesized oligonucleotide primer
taatacgactcactatagggagagccaccatgggctccagactcttcttt

SEQ ID NO: 49 - DNA, 50 bp, Artificial Sequence
  Artificially synthesized oligonucleotide primer
taatacgactcactatagggagagccaccatgtctaacactgtcctcgct

SEQ ID NO: 50 - DNA, 99 bp, Artificial Sequence
  Artificially synthesized oligonucleotide primer
ttttttttttttttttttttttttttttttttttttttttttttttttttttttttttttttttttctatgaattctttcttttgaccatagccatcac

SEQ ID NO: 51 - DNA, 50 bp, Artificial Sequence
  Artificially synthesized oligonucleotide primer
taatacgactcactatagggagagccaccatgaagaggctgctgtgttct

SEQ ID NO: 52 - DNA, 47 bp, Artificial Sequence
  Artificially synthesized oligonucleotide primer
taatacgactcactatagggagagccaccatgagctgcaggcttctc

SEQ ID NO: 53 - DNA, 52 bp, Artificial Sequence
  Artificially synthesized oligonucleotide primer
taatacgactcactatagggagagccaccatgaacagattcctgggaatatc

SEQ ID NO: 54 - protein, 9 aa, Artificial Sequence
  Artifically synthesized peptide
LLWNGPMAV

SEQ ID NO: 55 - protein, 9 aa, Artificial Sequence
  Artifically synthesized peptide
GILGFVFTL